European Patent Specification EP 3 426 305 B1, published May 7, 2025. Title: Stabilized Radiolabeled Anti-CD45 Immunoglobulin Compositions. Applicant: Actinium Pharmaceuticals. The sequence listing filed with the application follows.

SEQUENCE LISTING (14 sequences)

SEQ ID NO: 1 - protein, 111 aa, murine
DIALTQSPASLAVSLGQRATISCRASKSVSTSGYSYLHWYQQKPGQPPKLLIYLASNLESGVPARFSGSGSGTDFTLNIHPVEEEDAATYYCQHSRELPFTFGSGTKLEIK

SEQ ID NO: 2 - protein, 123 aa, murine
EVKLLESGGGLVQPGGSLKLSCAASGFDFSRYWMSWVRQAPGKGLEWIGEINPTSSTINFTPSLKDKVFISRDNAKNTLYLQMSKVRSEDTALYYCARGNYYRYGDAMDYWGQGTSVTVSSAK

SEQ ID NO: 3 - protein, 15 aa, murine
RASKSVSTSGYSYLH

SEQ ID NO: 4 - protein, 7 aa, murine
LASNLES

SEQ ID NO: 5 - protein, 9 aa, murine
QHSRELPFT

SEQ ID NO: 6 - protein, 10 aa, murine
GFDFSRYWMS

SEQ ID NO: 7 - protein, 17 aa, murine
EINPTSSTINFTPSLKD

SEQ ID NO: 8 - protein, 12 aa, murine
GNYYRYGDAMDY

SEQ ID NO: 9 - DNA, 717 bp, murine
atggagacagacacactcctgttatgggtactgctgctctgggttccaggttccactggtgacattgcgctgacacagtctcctgcttccttagctgtatctctgggacagagggccaccatctcatgcagggccagcaaaagtgtcagtacatctggctatagttatctgcactggtaccaacagaaaccaggacagccacccaaactcctcatctatcttgcatccaacctagaatctggggtccctgccaggttcagtggcagtgggtctgggacagacttcaccctcaacatccatcctgtggaggaggaggatgctgcaacctattactgtcagcacagtagggagcttccattcacgttcggctcggggacaaagttggaaataaaacgggctgatgctgcaccaactgtatccatcttcccaccatccagtgagcagttaacatctggaggtgcctcagtcgtgtgcttcttgaacaacttctaccccaaagacatcaatgtcaagtggaagattgatggcagtgaacgacaaaatggcgtcctgaacagttggactgatcaggacagcaaagacagcacctacagcatgagcagcaccctcacgttgaccaaggacgagtatgaacgacataacagctatacctgtgaggccactcacaagacatcaacttcacccattgtcaagagcttcaacaggaatgagtgttag

SEQ ID NO: 10 - DNA, 1389 bp, murine
atggattttgggctgattttttttattgttgctcttttaaaaggggtccagtgtgaggtgaagcttctcgagtctggaggtggcctggtgcagcctggaggatccctgaaactctcctgtgcagcctcaggattcgatttcagtagatactggatgagttgggtccggcaggctccagggaaagggctagaatggattggagagattaatccaactagcagtacgataaactttacgccatctctaaaggataaagtcttcatctccagagacaacgccaaaaatacgctgtacctgcaaatgagcaaagtgagatctgaggacacagccctttattactgtgcaagagggaactactataggtacggagatgctatggactactggggtcaaggaacctcagtcaccgtctcctcagccaaaacgacacccccatctgtctatccactggcccctggatctgctgcccaaactaactccatggtgaccctgggatgcctggtcaagggctatttccctgagccagtgacagtgacctggaactctggatccctgtccagcggtgtgcacaccttcccagctgtcctgcagtctgacctctacactctgagcagctcagtgactccctccagcacctggcccagcgagaccgtcacctgcaacgttgcccacccggccagcagcaccaaggtggacaagaaaattgtgcccagggattgtggttgtaagccttgcatatgtacagtcccagaagtatcatctgtcttcatcttccccccaaagcccaaggatgtgctcaccattactctgactcctaaggtcacgtgtgttgtggtagacatcagcaaggatgatcccgaggtccagttcagctggtttgtagatgatgtggaggtgcacacagctcagacgcaaccccgggaggagcagttcaacagcactttccgctcagtcagtgaacttcccatcatgcaccaggactggctcaatggcaaggagttcaaatgcagggtcaacagtgcagctttccctgcccccatcgagaaaaccatctccaaaaccaaaggcagaccgaaggctccacaggtgtacaccattccacctcccaaggagcagatggccaaggataaagtcagtctgacctgcatgataacagacttcttccctgaagacattactgtggagtggcagtggaatgggcagccagcggagaactacaagaacactcagcccatcatggacacagatggctcttacttcgtctacagcaagctcaatgtgcagaagagcaactgggaggcaggaaatactttcacctgctctgtgttacatgagggcctgcacaaccaccatactgagaagagcctctcccactctcctggtaaatga

SEQ ID NO: 11 - protein, 7 aa, murine
DIALTQS

SEQ ID NO: 12 - protein, 7 aa, murine
EVKLLES

SEQ ID NO: 13 - protein, 238 aa, murine
METDTLLLWVLLLWVPGSTGDIALTQSPASLAVSLGQRATISCRASKSVSTSGYSYLHWYQQKPGQPPKLLIYLASNLESGVPARFSGSGSGTDFTLNIHPVEEEDAATYYCQHSRELPFTFGSGTKLEIKRADAAPTVSIFPPSSEQLTSGGASVVCFLNNFYPKDINVKWKIDGSERQNGVLNSWTDQDSKDSTYSMSSTLTLTKDEYERHNSYTCEATHKTSTSPIVKSFNRNEC

SEQ ID NO: 14 - protein, 463 aa, murine
MDFGLIFFIVALLKGVQCEVKLLESGGGLVQPGGSLKLSCAASGFDFSRYWMSWVRQAPGKGLEWIGEINPTSSTINFTPSLKDKVFISRDNAKNTLYLQMSKVRSEDTALYYCARGNYYRYGDAMDYWGQGTSVTVSSAKTTPPSVYPLAPGSAAQTNSMVTLGCLVKGYFPEPVTVTWNSGSLSSGVHTFPAVLQSDLYTLSSSVTVPSSTWPSETVTCNVAHPASSTKVDKKIVPRDCGCKPCICTVPEVSSVFIFPPKPKDVLTITLTPKVTCVVVDISKDDPEVQFSWFVDDVEVHTAQTQPREEQFNSTFRSVSELPIMHQDWLNGKEFKCRVNSAAFPAPIEKTISKTKGRPKAPQVYTIPPPKEQMAKDKVSLTCMITDFFPEDITVEWQWNGQPAENYKNTQPIMDTDGSYFVYSKLNVQKSNWEAGNTFTCSVLHEGLHNHHTEKSLSHSPGK